European Patent Specification EP 3 725 878 B1, published April 1, 2026. Title: PHOSPHOLIPASE C AND ENCODING GENE THEREOF. Applicant: WILMAR (SHANGHAI) BIOTECHNOLOGY RESEARCH & DEVELOPMENT CENTER CO., LTD. The sequence listing filed with the application follows.

SEQUENCE LISTING (6 sequences)

SEQ ID NO: 1 - DNA, 738 bp, Artificial sequence
  Phospholipase C
tggtcagctgaggacaagcataaggaaggtgtgaatagtcacttatggatcgtgaaccgtgccattgatataatgtctaggaatacaactctggttaagcaagatagagttgctcaattgaatgaatggcgtacagagctagagaatggcatctacgctgctgatcatgaaaacccctattacgatgacagtaccttcgcttctcacttttacgatccagacaacggaaagacatatatcccattcgccaagcaagctaaggagactggagctaagtacttcaagttggctggagagtcatacaagaataaagacatgaagcaggccttcttttatcttgggttgtcattgcattatttgggcgatgtcaaccaacctatgcatgccgcatcctttacggacctgtcctatccacagggttttcactccaagtacgagaactttgtcgatactattaaagacaactacaaagttaccgatgggaacggatattggaattggaaaggcaccaaccctgaagaatggattcacggtgcagcagtagttgcaaaacaggactactctggaattgtcaatgacaataccaaagattggtttgtgaaagccgcagtctcccaggaatatgcagataaatggagagctgaagttacacctatgactggtaaacgactaatggatgcccaaagagttactgctggttacattcaattatggttcgacacttacggtgacaggtaa

SEQ ID NO: 2 - protein, 245 aa, Artificial sequence
  Phospholipase C
WSAEDKHKEGVNSHLWIVNRAIDIMSRNTTLVKQDRVAQLNEWRTELENGIYAADHENPYYDDSTFASHFYDPDNGKTYIPFAKQAKETGAKYFKLAGESYKNKDMKQAFFYLGLSLHYLGDVNQPMHAASFTDLSYPQGFHSKYENFVDTIKDNYKVTDGNGYWNWKGTNPEEWIHGAAVVAKQDYSGIVNDNTKDWFVKAAVSQEYADKWRAEVTPMTGKRLMDAQRVTAGYIQLWFDTYGDR

SEQ ID NO: 3 - DNA, 738 bp, Artificial sequence
  Phospholipase C
tggtcagctgaggacaagcataaggaagatgtgaatagtcacttatggatcgtgaaccgtgccattgatataatgtctaggaatacaactctggttaagcaagatagagttgctcaattgaatgaatggcgtacagagctagagaatggcatctacgctgctgatcatgaaaacccctattacgatgacagtaccttcgcttctcacttttacgatccagacaacggaaagacatatatcccattcgccaagcaagctaaggagactggagctaagtacttcaagttggctggagagtcatacaagaataaagacatgaagcaggccttcttttatcttgggttgtcattgcattatttgggcgatgtcaaccaacctatgcatgccgcatcctttacggacctgtcctatccacagggttttcactccaagtacgagaactttgtcgatactattaaagacaactacaaagttaccgatgggaacggatattggaattggaaaggcaccaaccctgaagaatggattcacggtgcagcagtagttgcaaaacaggactactctggaattgtcaatgacaataccaaagattggtttgtgaaagccgcagtctcccaggaatatgcagataaatggagagctgaagttacacctatgactggtaaacgactaatggatgcccaaagagttactgctggttacattcaattatggttcgacacttacggtgacaggtaa

SEQ ID NO: 4 - protein, 245 aa, Artificial sequence
  Phospholipase C
WSAEDKHKEDVNSHLWIVNRAIDIMSRNTTLVKQDRVAQLNEWRTELENGIYAADHENPYYDDSTFASHFYDPDNGKTYIPFAKQAKETGAKYFKLAGESYKNKDMKQAFFYLGLSLHYLGDVNQPMHAASFTDLSYPQGFHSKYENFVDTIKDNYKVTDGNGYWNWKGTNPEEWIHGAAVVAKQDYSGIVNDNTKDWFVKAAVSQEYADKWRAEVTPMTGKRLMDAQRVTAGYIQLWFDTYGDR

SEQ ID NO: 5 - DNA, 29 bp, Artificial sequence
  Forward primer
ctgaagcttggtcagctgaggacaagcat

SEQ ID NO: 6 - DNA, 38 bp, Artificial sequence
  Reverse primer
ccggaattcttacctgtcaccgtaagtgtcgaaccata